European Patent Application EP 4 407 040 A1, published July 31, 2024. Title: 褐色脂肪細胞を用いたスクリーニング方法. Applicant: 株式会社片岡製作所. The sequence listing filed with the application follows.

SEQUENCE LISTING (12 sequences)

SEQ ID NO: 1 - DNA, 23 bp, synthetic construct
  misc_feature 1..23: note = Synthesized oligonucleotide to act as a PCR sense primer to amplify Tbp gene.
  source 1..23: mol_type = other DNA
actacggggttatcacctgtgag

SEQ ID NO: 2 - DNA, 22 bp, synthetic construct
  misc_feature 1..22: note = Synthesized oligonucleotide to act as a PCR antisense primer to amplify Tbp gene.
  source 1..22: mol_type = other DNA
gtgcaggagtaggccacattac

SEQ ID NO: 3 - DNA, 20 bp, synthetic construct
  misc_feature 1..20: note = Synthesized oligonucleotide to act as a PCR sense primer to amplify Ucp1 gene.
  source 1..20: mol_type = other DNA
tctacgacacggtccaggag

SEQ ID NO: 4 - DNA, 22 bp, synthetic construct
  misc_feature 1..22: note = Synthesized oligonucleotide to act as a PCR antisense primer to amplify Ucp1 gene.
  source 1..22: mol_type = other DNA
gaatactgccactcctccagtc

SEQ ID NO: 5 - DNA, 21 bp, synthetic construct
  misc_feature 1..21: note = Synthesized oligonucleotide to act as a PCR sense primer to amplify Fabp4 gene.
  source 1..21: mol_type = other DNA
gccaggaatttgacgaagtca

SEQ ID NO: 6 - DNA, 22 bp, synthetic construct
  misc_feature 1..22: note = Synthesized oligonucleotide to act as a PCR antisense primer to amplify Fabp4 gene.
  source 1..22: mol_type = other DNA
cccatttctgcacatgtaccag

SEQ ID NO: 7 - DNA, 24 bp, synthetic construct
  misc_feature 1..24: note = Synthesized oligonucleotide to act as a PCR sense primer to amplify Cidea gene.
  source 1..24: mol_type = other DNA
aaggccaccatgtatgagatgtac

SEQ ID NO: 8 - DNA, 20 bp, synthetic construct
  misc_feature 1..20: note = Synthesized oligonucleotide to act as a PCR antisense primer to amplify Cidea gene.
  source 1..20: mol_type = other DNA
acaggaaccgcagcagactc

SEQ ID NO: 9 - DNA, 21 bp, synthetic construct
  misc_feature 1..21: note = Synthesized oligonucleotide to act as a PCR sense primer to quantify mtDNA.
  source 1..21: mol_type = other DNA
acaccctcctagccttactac

SEQ ID NO: 10 - DNA, 19 bp, synthetic construct
  misc_feature 1..19: note = Synthesized oligonucleotide to act as a PCR antisense primer to quantify mtDNA.
  source 1..19: mol_type = other DNA
gatatagggtcgaagccgc

SEQ ID NO: 11 - DNA, 18 bp, synthetic construct
  misc_feature 1..18: note = Synthesized oligonucleotide to act as a PCR sense primer to quantify NuDNA.
  source 1..18: mol_type = other DNA
agggtatctgggctctgg

SEQ ID NO: 12 - DNA, 21 bp, synthetic construct
  misc_feature 1..21: note = Synthesized oligonucleotide to act as a PCR antisense primer to quantify NuDNA.
  source 1..21: mol_type = other DNA
ggctgaaaagctcccgattat